European Patent Application EP 4 371 578 A1, published May 22, 2024. Title: Composition comprising hyaluronic acid complex for preventing or treating skin disease. Applicant: AJOU UNIVERSITY INDUSTRY-ACADEMIC COOPERATION FOUNDATION. The sequence listing filed with the application follows.

SEQUENCE LISTING (16 sequences)

SEQ ID NO: 1 - DNA, 20 bp, Artificial Sequence
  source 1..20: mol_type = other DNA
tgcaccaccaactgcttagc

SEQ ID NO: 2 - DNA, 21 bp, Artificial Sequence
  source 1..21: mol_type = other DNA
ggcatggactgtggtcatgag

SEQ ID NO: 3 - DNA, 20 bp, Artificial Sequence
  source 1..20: mol_type = other DNA
tgggatcattgccctgtgag

SEQ ID NO: 4 - DNA, 20 bp, Artificial Sequence
  source 1..20: mol_type = other DNA
ccaggtttcgaagtggtggt

SEQ ID NO: 5 - DNA, 20 bp, Artificial Sequence
  source 1..20: mol_type = other DNA
ccactcacctcttcagaacg

SEQ ID NO: 6 - DNA, 22 bp, Artificial Sequence
  source 1..22: mol_type = other DNA
catctttggaaggttcaggttg

SEQ ID NO: 7 - DNA, 22 bp, Artificial Sequence
  source 1..22: mol_type = other DNA
ttcgacacatgggataacgagg

SEQ ID NO: 8 - DNA, 21 bp, Artificial Sequence
  source 1..21: mol_type = other DNA
tttttgctgtgagtcccggag

SEQ ID NO: 9 - DNA, 22 bp, Artificial Sequence
  source 1..22: mol_type = other DNA
aaccctgaccatccaagtcaaa

SEQ ID NO: 10 - DNA, 22 bp, Artificial Sequence
  source 1..22: mol_type = other DNA
cttggcctcgcatcttagaaag

SEQ ID NO: 11 - DNA, 23 bp, Artificial Sequence
  source 1..23: mol_type = other DNA
gcttacaaactcggtgaacaact

SEQ ID NO: 12 - DNA, 21 bp, Artificial Sequence
  source 1..21: mol_type = other DNA
gtggaatctctgcccacttcc

SEQ ID NO: 13 - DNA, 23 bp, Artificial Sequence
  source 1..23: mol_type = other DNA
atgctgactatggctacaaaagc

SEQ ID NO: 14 - DNA, 19 bp, Artificial Sequence
  source 1..19: mol_type = other DNA
tcgggcaatcatcaggcac

SEQ ID NO: 15 - DNA, 24 bp, Artificial Sequence
  source 1..24: mol_type = other DNA
gaaagcagttagcaaggaaaggtc

SEQ ID NO: 16 - DNA, 23 bp, Artificial Sequence
  source 1..23: mol_type = other DNA
atgtagggaagtgatgggagagg